European Patent Application EP 4 265 641 A1, published October 25, 2023. Title: Development and application of complement inhibitor. Applicant: Keymed Biosciences Co.,Ltd. The sequence listing filed with the application follows.

SEQUENCE LISTING (216 sequences)

SEQ ID NO: 1 - protein, 397 aa, Homo sapiens
HHHHHHASQPCPYPMAPPNGHVSPVQAKYILKDSFSIFCETGYELLQGHLPLKSFTAVCQKDGSWDRPMPACSIVDCGPPDDLPSGRVEYITGPGVTTYKAVIQYSCEETFYTMKVNDGKYVCEADGFWTSSKGEKSLPVCEPVCGLSARTTGGRIYGGQKAKPGDFPWQVLILGGTTAAGALLYDNWVLTAAHAVYEQKHDASALDIRMGTLKRLSPHYTQAWSEAVFIHEGYTHDAGFDNDIALIKLNNKVVINSNITPICLPRKEAESFMRTDDIGTASGWGLTQRGFLARNLMYVDIPIVDHQKCTAAYEKPPYPRGSVTANMLCAGLESGGKDSCRGDAGGALVFLDSETERWFVGGIVSWGSMNCGEAGQYGVYTKVINYIPWIENIISDF

SEQ ID NO: 2 - protein, 397 aa, Macaca fascicularis
HHHHHHASQPCPYPMAPPNGHLSPVQAKYILKDSFSIFCEPGYELLQGHLPLKSFAAVCQKDGSWDQPMPSCSIVDCGPPDDLPSGRVEYITGPEVTTYKAVIQYSCEETFYTMKVNDGKYVCEADGFWTSSKGERSPPVCEPVCGLSARTTGGRIYGGQKAKPGDFPWQVLILGGSTAAGALLYDNWVLTAAHAIYEQKHDASSLDIRLGALKRLSPHYTQAWAEAVFIHEGYTHDAGFDNDIALIKLNNKVVINSNITPICLPRKEAESFMRTDDIGTASGWGLTQRGLLARNLMYVDIPIVDHQKCTAAYEKPPYSGGSVTANMLCAGLESGGKDSCRGDAGGALVFLDNETQRWFVGGIVSWGSMNCGEAGQYGVYTKVINYIPWIKNIISNF

SEQ ID NO: 3 - protein, 396 aa, Mus musculus
HHHHHHASRPCPDPTAPPNGSISPVQAIYVLKDRFSVFCKTGFELLQGSVPLKSFTAVCQKDGSWDRPMPECSIIDCGPPDDLPNGHVDYITGPEVTTYKAVIQYSCEETFYTMSSNGKYVCEADGFWTSSKGEKLPPVCEPVCGLSTHTIGGRIVGGQPAKPGDFPWQVLLLGQTTAAAGALIHDNWVLTAAHAVYEKRMAASSLNIRMGILKRLSPHYTQAWPEEIFIHEGYTHGAGFDNDIALIKLKNKVTINGSIMPVCLPRKEAASLMRTDFTGTVAGWGLTQKGLLARNLMFVDIPIADHQKCTAVYEKLYPGVRVSANMLCAGLETGGKDSCRGDAGGALVFLDNETQRWFVGGIVSWGSINCGAADQYGVYTKVINYIPWIENIISNF

SEQ ID NO: 4 - protein, 396 aa, Rattus norvegicus
HHHHHHASQPCPDPTAPPNGHISPVQATYVLKDSFSVFCKTGFELLQGSVPLKSFTAVCQKDGSWDRPIPECSIIDCGPPDDLPNGHVDYITGPEVTTYKAVIQYSCEETFYTMSSNGKYVCEADGFWTSSKGEKSLPVCKPVCGLSTHTSGGRIIGGQPAKPGDFPWQVLLLGETTAAGALIHDDWVLTAAHAVYGKTEAMSSLDIRMGILKRLSLIYTQAWPEAVFIHEGYTHGAGFDNDIALIKLKNKVTINRNIMPICLPRKEAASLMKTDFVGTVAGWGLTQKGFLARNLMFVDIPIVDHQKCATAYTKQPYPGAKVTVNMLCAGLDRGGKDSCRGDAGGALVFLDNETQRWFVGGIVSWGSINCGGSEQYGVYTKVTNYIPWIENIINNF

SEQ ID NO: 5 - protein, 114 aa, Mus musculus
DVQLQESGPGLVKPSQSLSLTCTVTGYSITSDYAWNWIRQFSGDKLEWMGYISYSGSTSYNPSLKSRISITRDTSKNQFFLHLSSVTTEDTATYFCARYWGDYWGHGTTLTVSS

SEQ ID NO: 6 - DNA, 342 bp, Mus musculus
gatgtgcagcttcaggagtcgggacctggcctggtgaaaccttctcagtctctgtccctcacctgcactgtcactggctactcaatcaccagtgattatgcctggaactggatccggcagttttcaggagacaaactggagtggatgggctacataagctacagtggttccactagctataacccatctctcaaaagtcgaatctctatcactcgagacacatccaagaaccagttcttcctgcacttgagttctgtgactactgaggacacagccacatatttctgtgcaagatattggggcgactactggggccacggcaccactctcacagtctcctca

SEQ ID NO: 7 - protein, 7 aa, Mus musculus
TSDYAWN

SEQ ID NO: 8 - protein, 16 aa, Mus musculus
YISYSGSTSYNPSLKS

SEQ ID NO: 9 - protein, 5 aa, Mus musculus
YWGDY

SEQ ID NO: 10 - protein, 107 aa, Mus musculus
DSVMTQSQKFMSTSVGDRVSVTCKASHNVGTNVAWFQQKPGQSPKGLIYSASYRSSGVPDRFTGSGSGTDFTLTISNVQSEDLAEYFCLQYNSNPLTFGGGTKLEVK

SEQ ID NO: 11 - DNA, 321 bp, Mus musculus
gacagtgtgatgacccagtctcaaaaattcatgtccacatcagtaggagacagggtcagcgtcacctgcaaggccagtcacaatgtgggtactaatgtagcctggtttcaacagaaaccaggacaatctcctaaaggactgatttactcggcatcctaccggtccagtggagtccctgatcgcttcacaggcagtggatctgggacagacttcactctcaccatcagcaatgtgcagtctgaagacttggcagagtatttctgtctacaatataacagcaatcctctgacgttcggtggaggcaccaagctggaggtcaag

SEQ ID NO: 12 - protein, 11 aa, Mus musculus
KASHNVGTNVA

SEQ ID NO: 13 - protein, 7 aa, Mus musculus
SASYRSS

SEQ ID NO: 14 - protein, 9 aa, Mus musculus
LQYNSNPLT

SEQ ID NO: 15 - protein, 118 aa, Mus musculus
DVQLQESGPGLVRPSQSLSLTCTVTGYSITSDYAWNWIRQFPGNKLEWMGYISYSGRTSYNPSLKSRLSITRDTSKNQFFLQLNSVSSADTATYYCAIISTAVDFDYWGQGTTLTVSS

SEQ ID NO: 16 - DNA, 354 bp, Mus musculus
gatgtacaacttcaggagtcgggacctggcctggtgagaccttctcagtctctgtccctcacctgcactgtcactggctactcaatcaccagtgattatgcctggaactggatccggcagtttccaggaaacaaactggagtggatgggctacataagttacagtggtcgcactagttacaacccctctctcaaaagtcgactctctatcactcgagacacatccaagaaccagttcttcctgcagttgaattctgtgagttctgcggacacagccacgtattactgtgcaattatttctacggcagtagactttgactactggggccaaggcaccactctcacagtctcctca

SEQ ID NO: 17 - protein, 16 aa, Mus musculus
YISYSGRTSYNPSLKS

SEQ ID NO: 18 - protein, 9 aa, Mus musculus
ISTAVDFDY

SEQ ID NO: 19 - protein, 108 aa, Mus musculus
QTVLTQSPAIMSASLGERVTMTCTASSSVSSSYLLWYQQKPGSSPKLWIYSTSKLASGVPVRFSGSGSGTSYSLTISSMEADDAATYYCLQYNRSPLTFGAGTKLELK

SEQ ID NO: 20 - DNA, 324 bp, Mus musculus
caaactgttctcacccagtctccagcaatcatgtctgcatctctaggggaacgggtcaccatgacctgcactgccagctcaagtgtaagttccagttacttgctctggtaccagcagaagccaggatcctcccccaaactctggatttatagcacatccaagttggcttctggagtcccagttcgcttcagtggcagtgggtctgggacctcttactctctcacaatcagcagcatggaggctgacgatgctgccacttattactgcctccagtataatcgttccccgctcacgttcggtgctgggaccaagctggagctgaaa

SEQ ID NO: 21 - protein, 12 aa, Mus musculus
TASSSVSSSYLL

SEQ ID NO: 22 - protein, 7 aa, Mus musculus
STSKLAS

SEQ ID NO: 23 - protein, 9 aa, Mus musculus
LQYNRSPLT

SEQ ID NO: 24 - protein, 117 aa, Mus musculus
EVQLQESGPGLVKPSQSLSLACTVTGYSITSDYAWHWIRQFPGNKLEWMGFISYSGRTNYNPPLTSRISITRDTSKNQFFLQLNSVTTEDTATYYCARSYDYWFGYWGQGTLVTVSA

SEQ ID NO: 25 - DNA, 351 bp, Mus musculus
gaggtccagctgcaggagtcgggacctggcctggtgaaaccttctcagtctctgtccctcgcctgcactgtcactggctactcaatcaccagtgattatgcctggcactggatccggcagtttccaggaaacaaactggagtggatgggcttcataagctacagtggtagaactaactacaacccacctctcacaagtcgaatctctatcactcgagacacatccaagaaccagttcttcctgcagttgaattctgtgactactgaggacacagccacatattactgtgcaagatcatatgattactggtttggttattggggccaagggactctggtcactgtctctgca

SEQ ID NO: 26 - protein, 7 aa, Mus musculus
TSDYAWH

SEQ ID NO: 27 - protein, 16 aa, Mus musculus
FISYSGRTNYNPPLTS

SEQ ID NO: 28 - protein, 8 aa, Mus musculus
SYDYWFGY

SEQ ID NO: 29 - protein, 112 aa, Mus musculus
NVLMTQTPLSLPVSLGDQASISCRSSQSLVHSNGNTYLEWYMQKPGQSPKLLIYTVSRRFSGVPDRFSGSGSGTDFTLKISRVEAEDLGVYYCFQGSHVPVTFGAGTKLELK

SEQ ID NO: 30 - DNA, 336 bp, Mus musculus
aatgttttgatgacccaaactccactctccctgcctgtcagtcttggagatcaagcctccatctcttgcagatctagtcagagtcttgtacatagtaatggaaacacctatttagaatggtacatgcagaaaccaggccagtctccaaagctcctgatctacacagtttccagacgattttctggggtcccagacaggttcagtggcagtggatcagggacagatttcacactcaagatcagcagagtggaggctgaggatctgggagtttattattgctttcaaggttcacatgttccggtcacgttcggtgctgggaccaagctggagctgaaa

SEQ ID NO: 31 - protein, 16 aa, Mus musculus
RSSQSLVHSNGNTYLE

SEQ ID NO: 32 - protein, 7 aa, Mus musculus
TVSRRFS

SEQ ID NO: 33 - protein, 9 aa, Mus musculus
FQGSHVPVT

SEQ ID NO: 34 - protein, 117 aa, Mus musculus
DVQLQESGPGLVKPSQSLSLTCTVTGYSITSDYAWKWIRQFPGNKLEWMGYISYSGSTSYNPSLKGRISITRDTSKNQFFLHLQSVTIEDTATYYCAILGYFAMDYWGQGTPVTVSS

SEQ ID NO: 35 - DNA, 351 bp, Mus musculus
gatgtacaacttcaggagtcgggacctggcctggtgaaaccttctcagtctctgtccctcacctgcactgtcactggctactcaatcaccagtgattatgcctggaagtggatccggcagtttccaggaaacaaactggagtggatgggctacataagttacagtggcagcactagctacaacccttctctcaaaggtcgaatctctatcactcgagacacatccaagaaccagtttttcctgcacttgcaatctgtgactattgaggacacagccacctattactgtgcaatactaggttactttgctatggactactgggggcaaggaaccccagtcaccgtctcctca

SEQ ID NO: 36 - protein, 7 aa, Mus musculus
TSDYAWK

SEQ ID NO: 37 - protein, 16 aa, Mus musculus
YISYSGSTSYNPSLKG

SEQ ID NO: 38 - protein, 8 aa, Mus musculus
LGYFAMDY

SEQ ID NO: 39 - protein, 107 aa, Mus musculus
DIVMTQSQKFMSTSVGDRVSITCKASQNVRVDVAWYQQKSGQSPKSLIYLASNRHTGVPDRFTGSGSGTDFTLTISNVQSEDLADYFCLQHWSYPLTFGGGTKLEIK

SEQ ID NO: 40 - DNA, 321 bp, Mus musculus
gacattgtgatgacccagtctcaaaaattcatgtccacttcagtaggagacagggtcagcatcacctgcaaggccagtcagaatgttcgtgttgacgttgcctggtatcaacagaaatcagggcagtctcctaaatcactgatttacttggcatccaaccggcacactggagtccctgatcgcttcacaggcagtggatctgggacagatttcactctcaccattagcaatgtgcaatctgaagacctggcagattatttctgtctacaacattggagttatcctctgacgttcggtggaggcaccaagctggaaatcaaa

SEQ ID NO: 41 - protein, 11 aa, Mus musculus
KASQNVRVDVA

SEQ ID NO: 42 - protein, 7 aa, Mus musculus
LASNRHT

SEQ ID NO: 43 - protein, 9 aa, Mus musculus
LQHWSYPLT

SEQ ID NO: 44 - protein, 118 aa, Mus musculus
DVQLQESGPGLVKPSQSLSLTCTVTGYSITSDYAWNWIRQFPGNTLEWMGYISYSGRTSYNPSLIGRISITRDTTKNQFFLQLNSVSTEDTATYYCAKLAGGHGMDYWGQGTSVTVSS

SEQ ID NO: 45 - DNA, 354 bp, Mus musculus
gatgtgcagcttcaggagtcgggacctggcctggtgaaaccttctcagtctctgtccctcacctgcactgtcactggctactcaatcaccagtgattatgcctggaactggatccggcagtttccaggaaacacattggagtggatgggctatataagttatagtggtaggactagctacaacccatctctgataggtcgaatctcaatcactcgagacacaaccaagaaccagttctttctgcagttgaattctgtgtctactgaggacacagccacatattactgtgcaaaattggccggaggacatgggatggactactggggtcaaggaacctcagtcaccgtctcctca

SEQ ID NO: 46 - protein, 16 aa, Mus musculus
YISYSGRTSYNPSLIG

SEQ ID NO: 47 - protein, 9 aa, Mus musculus
LAGGHGMDY

SEQ ID NO: 48 - protein, 106 aa, Mus musculus
NIVMTQSQQFMSTSVGDRVSVTCKASQNVDTNVAWYQQKPGQSPKALIYSASYRYSGVPDRFTGSGSGTDFTLTISNVQSEDLAEYFCLQYNSYLTFGSGTKLELK

SEQ ID NO: 49 - DNA, 318 bp, Mus musculus
aacattgtgatgacccagtctcaacaattcatgtccacatcagtaggagacagggtcagcgtcacctgcaaggccagtcagaatgtggatactaatgtagcctggtatcaacagaaaccaggacaatctcctaaagcactgatttactcggcatcctaccggtacagtggagtccctgatcgcttcacaggcagtggatctgggacagatttcactctcaccatcagcaatgtgcagtctgaagacttggcagaatatttctgtctgcaatataatagttacctcacgttcggttctgggaccaagctggagctgaaa

SEQ ID NO: 50 - protein, 11 aa, Mus musculus
KASQNVDTNVA

SEQ ID NO: 51 - protein, 7 aa, Mus musculus
SASYRYS

SEQ ID NO: 52 - protein, 8 aa, Mus musculus
LQYNSYLT

SEQ ID NO: 53 - protein, 118 aa, Mus musculus
DVQLQESGPGLVRPSQSLSLTCTVTGYSITSDYAWNWIRQFPGNKLEWMGYISYSGRTSYNPSLKSRLSVTRDTSKNQFFLQLNSVNAADTATYYCAIISTAVDFDYWGQGTTLTVSS

SEQ ID NO: 54 - DNA, 354 bp, Mus musculus
gatgtacaacttcaggagtcgggacctggcctggtgagaccttctcagtctctgtccctcacctgcactgtcactggctactcaatcaccagtgattatgcctggaactggatccggcagtttccaggaaacaaactggagtggatgggctacataagttacagtggtcgcactagctacaacccctctctcaagagtcgactctctgtcactcgagacacatccaagaaccagttcttcctgcagttgaattctgtgaatgctgcggacacagccacgtattactgtgcaattatttctacggcagtagactttgactactggggccaaggcaccactctcacagtctcctca

SEQ ID NO: 55 - protein, 108 aa, Mus musculus
QIVLTQSPAIMSASLGERVTMTCTASSSVSSSYLLWYQQKPGSSPKLWIYSSSKLASGVPVRFSGSGSGTSYSLTISSMEAEDAATYYCLQYNRSPLTFGAGTKLELK

SEQ ID NO: 56 - DNA, 324 bp, Mus musculus
caaattgttctcacccagtctccagcaatcatgtctgcatctctaggggaacgggtcaccatgacctgcactgccagctcaagtgtaagttccagttacttgctctggtaccagcagaagccaggatcctcccccaaactctggatttatagctcatccaagttggcttctggagtcccagttcgcttcagtggcagtgggtctgggacctcttactctctcacaatcagcagcatggaggctgaagatgctgccacttattactgcctccagtataatcgttccccgctcacgttcggtgctgggaccaagctggagctgaaa

SEQ ID NO: 57 - protein, 7 aa, Mus musculus
SSSKLAS

SEQ ID NO: 58 - protein, 118 aa, Mus musculus
DVQLQESGPGLVKPSQSLSLTCTVTGYSITSDYAWNWIRQFPGNKLEWMGYISYSGRTSYNPSLKSRISITRDTSKNQFFLQLNSVTTEDTATYYCAKLGGGHGMDYWGQGTSVTVSS

SEQ ID NO: 59 - DNA, 354 bp, Mus musculus
gatgtgcagcttcaggagtcgggacctggcctggtgaaaccttctcagtctctgtccctcacctgcactgtcactggctactcaatcaccagtgattatgcctggaactggatccggcagtttccaggaaacaaattggagtggatgggctacataagttatagtggtaggactagctacaacccatctctgaaaagtcgaatctcaatcactcgagacacatccaagaaccagttcttcctgcagttgaattctgtgactactgaggacacagccacatattactgtgcaaaattgggcggaggacatgggatggactactggggtcaaggaacctcagtcaccgtctcctca

SEQ ID NO: 60 - protein, 9 aa, Mus musculus
LGGGHGMDY

SEQ ID NO: 61 - protein, 105 aa, Mus musculus
IVMTQSQKFMSTSVGDRVSVTCKASQNVDTNVAWYQQKPGQSPKALIYSASYRYSGVPDRFTGSGSGTDFTLTISNVQSEDLAEYFCLQYNSYLTFGSGTKLELK

SEQ ID NO: 62 - DNA, 317 bp, Mus musculus
acattgtgatgacccagtctcaaaaattcatgtccacatcagtaggagacagggtcagcgtcacctgcaaggccagtcagaatgtggatactaatgtagcctggtatcaacagaaaccagggcaatctcctaaagcgctgatttactcggcatcctaccgttacagtggagtccctgatcgcttcacaggcagtggatctgggacagatttcactctcaccatcagcaatgtgcagtctgaagacttggcagagtatttctgtctgcaatataacagctacctcacgttcggttctgggaccaagctggagctgaaa

SEQ ID NO: 63 - protein, 120 aa, Mus musculus
QVTLKESGPGILKPSQTLILTCSFSGFSLNTSGMGVGWIRQPSGKGLEWLAHIWWDDDKDYNPSLKSQVTISKDTSTNQVFLKITSVDTADGATYYCVRDTTFLDAMDYWGQGTSVTVSS

SEQ ID NO: 64 - DNA, 360 bp, Mus musculus
caagttactctaaaagagtctggccctgggatattgaagccctcacagaccctcattctgacttgttctttctctgggttttcactgaacacttctggtatgggtgtaggctggattcgtcagccttcagggaagggtctggagtggctggcacacatttggtgggatgatgataaggactataacccatccctgaagagccaagtcacaatctccaaggatacctccacaaaccaggtgttcctcaagatcaccagtgtggacactgcagatggtgccacttactactgtgttcgagatactacgtttttagatgctatggactactggggtcaaggaacctcagtcaccgtctcctca

SEQ ID NO: 65 - protein, 8 aa, Mus musculus
NTSGMGVG

SEQ ID NO: 66 - protein, 16 aa, Mus musculus
HIWWDDDKDYNPSLKS

SEQ ID NO: 67 - protein, 10 aa, Mus musculus
DTTFLDAMDY

SEQ ID NO: 68 - protein, 112 aa, Mus musculus
DVLMTQTPLSLPVSLGDQASISCRSSQSIVHRNGNTFLEWYLQKPGQSPKLLIYRVSNRFSGVPDRFSGSGSGTDFTLKISRVEAEDLGVYYCFQGSHVPFTFGSGTKLEIK

SEQ ID NO: 69 - DNA, 336 bp, Mus musculus
gatgttttgatgacccaaactccactctccctgcctgtcagtcttggagatcaagcctccatctcttgcaggtctagtcagagcattgtacatcgtaatggaaacacctttttagaatggtacctgcagaaaccaggccagtctccaaagctcctgatctacagggtttccaaccgattttctggggtcccagacaggttcagtggcagtggatcagggacagatttcacactcaagatcagcagagtggaggctgaggatctgggagtttattactgctttcaaggttcacatgttccattcacgttcggctcggggacaaagttggaaataaaa

SEQ ID NO: 70 - protein, 16 aa, Mus musculus
RSSQSIVHRNGNTFLE

SEQ ID NO: 71 - protein, 7 aa, Mus musculus
RVSNRFS

SEQ ID NO: 72 - protein, 9 aa, Mus musculus
FQGSHVPFT

SEQ ID NO: 73 - protein, 118 aa, Mus musculus
DVQLQESGPGLVKPSQSLSLTCTVTGYSITSDYAWNWIRQLPGNKLEWVGYISYSGRTSYNPSLKSRISITRDTTKNQFFLQLNSVTTEDTATYYCAKLAGGHGMDYWGQGTSVTVSS

SEQ ID NO: 74 - DNA, 354 bp, Mus musculus
gatgtgcagcttcaggagtcgggacctggcctggtgaaaccttctcagtctctgtccctcacctgcactgtcactggctactcaatcaccagtgattatgcctggaactggatccggcagttaccaggaaacaaattggagtgggtgggctatataagttatagtggtaggactagctacaacccatctctgaaaagtcgaatctcaatcactcgagacacaaccaagaaccagttcttcctgcagttgaattctgtgactactgaggacacagccacatattactgtgcaaagttggccgggggacatgggatggactactggggtcaaggaacctcagtcaccgtctcctca

SEQ ID NO: 75 - protein, 106 aa, Mus musculus
NIVMTQSQKFMSTSVGDRVSVTCKASQNVDTNVAWYQQKPGQSPKALIHSASYRYSGVPDRFTGSGSGTDFILTISNVQSEDLAEYFCLQYNSYLTFGSGTKLELK

SEQ ID NO: 76 - DNA, 318 bp, Mus musculus
aacattgtgatgacccagtctcaaaaattcatgtccacatcagtaggagacagggtcagcgtcacctgcaaggccagtcagaatgtggatactaatgtagcctggtatcaacagaaaccagggcaatctcctaaagcactgattcactcggcatcctaccggtacagtggagtccctgatcgcttcacaggcagtggatctgggacagatttcattctcaccatcagtaatgtgcagtctgaagacttggcagagtatttctgtctgcaatataacagctacctcacgttcggttctgggaccaagctggagctgaaa

SEQ ID NO: 77 - protein, 116 aa, Mus musculus
DVQLQESGPGLVKPSQSLSLTCTVTGYSITSDYAWNWIRQFPGNKLEWMGYISYSGRTSYNPSLKSRISITRDTSKNQFFLHLNSVTTEDTATYFCAVLGLYFDYWGQGTPLTVSS

SEQ ID NO: 78 - DNA, 348 bp, Mus musculus
gatgtgcagcttcaggagtcgggacctggcctggtgaaaccttctcagtctctgtccctcacctgcactgtcactggctactcaatcaccagtgattatgcctggaactggatccggcagtttccaggaaacaaactggagtggatgggctacataagctacagtggtagaactagctacaacccatctctcaaaagtcgaatctctatcactcgagacacatccaagaaccagttcttcctgcacttgaattctgtgactactgaggacacagccacatatttctgtgcagtactgggactctactttgactactggggccaaggcacccctctcacagtctcctca

SEQ ID NO: 79 - protein, 7 aa, Mus musculus
LGLYFDY

SEQ ID NO: 80 - protein, 107 aa, Mus musculus
DIVMTQSQKFMSTSVGDRVSVTCKASQNVDTNVAWYQQKPGQSPKALIYSASYRYSGVPDRFTGSGSGTDFTLTISNVQSEDLAEYFCHQFNSNPLTFGAGTKLELK

SEQ ID NO: 81 - DNA, 321 bp, Mus musculus
gacattgtgatgacccagtctcaaaaattcatgtccacatcagtaggagacagggtcagcgtcacctgcaaagccagtcagaatgtggatactaatgtagcctggtatcaacagaaaccagggcaatctcctaaagcactgatttactcggcatcctaccggtacagtggagtccctgatcgcttcacaggcagtggatctgggacagatttcactctcaccatcagcaatgtgcagtctgaagacttggcagaatatttctgtcaccaatttaacagcaatcctctcacgttcggtgctgggaccaagctggagctgaaa

SEQ ID NO: 82 - protein, 9 aa, Mus musculus
HQFNSNPLT

SEQ ID NO: 83 - protein, 117 aa, Mus musculus
DVQLQESGPGLVKPSQSLSLTCTVTGYSITSDYAWKWIRQFPGNKLEWMGYISYSGSTSYHPSLKGRISITRDTSKNQFFLQLNSVTADDTATYYCAILGYYAMDYWGQGTSVTVSS

SEQ ID NO: 84 - DNA, 351 bp, Mus musculus
gatgtgcagcttcaggagtcgggacctggcctggtgaaaccttctcagtctctgtccctcacctgcactgtcactggctactcaatcaccagtgattatgcctggaaatggatccggcagtttccaggaaacaaactggaatggatgggctacataagctacagtggttccactagctatcacccatctctcaaaggtcgaatctccatcactcgagacacatccaagaaccagttcttcctgcagttgaattctgtgactgctgacgacacagccacatattactgtgcaatattaggttactatgctatggactactggggtcaaggaacctcagtcaccgtctcctca

SEQ ID NO: 85 - protein, 16 aa, Mus musculus
YISYSGSTSYHPSLKG

SEQ ID NO: 86 - protein, 8 aa, Mus musculus
LGYYAMDY

SEQ ID NO: 87 - protein, 107 aa, Mus musculus
DIVMTQSQKFMSTSVGDRVSITCKASQNVRVDVAWYQQKSGQSPRALIYLASNRHTGVPDRFTGSGSGTDFTLTITNVQSEDLADYFCLQHWSYPLTFGGGTKLEIK

SEQ ID NO: 88 - DNA, 321 bp, Mus musculus
gacattgtgatgacccagtctcaaaaattcatgtccacatcagtaggagacagggtcagtatcacctgcaaggccagtcagaatgttcgtgttgacgtagcctggtatcaacagaaatcagggcagtctcctagagcactgatttacttggcatccaaccggcacactggagtccctgatcgcttcacaggcagtggatctgggacagatttcactctcaccattaccaatgtgcaatctgaggacctggcagattatttctgtctacaacattggagttatcctctgacgttcggtggaggcaccaagctggaaatcaaa

SEQ ID NO: 89 - protein, 107 aa, Mus musculus
DIVMTQSQKFMSTSVGDRVSITCKASQNVRVDVAWYQQKSGQSPRALIYLASNRHTGVPDRFTGSGSGTDFTLTITNVQSEDLADYFCPQHWSYPLTFGGGTKLEIK

SEQ ID NO: 90 - DNA, 321 bp, Mus musculus
gacattgtgatgacccagtctcaaaaattcatgtccacatcagtaggagacagggtcagtatcacctgcaaggccagtcagaatgttcgtgttgacgtagcctggtatcaacagaaatcagggcagtctcctagagcactgatttacttggcatccaaccggcacactggagtccctgatcgcttcacaggcagtggatctgggacagatttcactctcaccattaccaatgtgcaatctgaggacctggcagattatttctgtccacaacattggagttatcctctgacgttcggtggaggcaccaagctggaaatcaaa

SEQ ID NO: 91 - protein, 9 aa, Mus musculus
PQHWSYPLT

SEQ ID NO: 92 - protein, 119 aa, Mus musculus
KVKLVESGGDLVKPGGSLKISCTASGFTFSNYAMSWIRQTPDKRLEWVATVSSGGPYTYYPDSVKGRFTISRDNAENTLYLQMSSLRSDDTAIYYCARQIYSDYDVTYWGQGTLVTVSA

SEQ ID NO: 93 - DNA, 357 bp, Mus musculus
aaagtgaagctggtggagtctgggggagacttagtgaagcctggagggtccctgaaaatctcctgtacagcctctggattcactttcagtaactatgccatgtcttggattcgccagactccggacaagaggctggagtgggtcgcaaccgttagtagtggtggtccttacacctactatccagacagtgtgaaggggcgattcaccatctccagagacaatgccgaaaacaccctgtacctgcaaatgagcagtctgaggtctgatgacacggccatatattactgtgcaaggcagatctactctgattacgacgtcacttactggggccaagggactctggtcactgtctctgca

SEQ ID NO: 94 - protein, 6 aa, Mus musculus
SNYAMS

SEQ ID NO: 95 - protein, 17 aa, Mus musculus
TVSSGGPYTYYPDSVKG

SEQ ID NO: 96 - protein, 10 aa, Mus musculus
QIYSDYDVTY

SEQ ID NO: 97 - protein, 106 aa, Mus musculus
QIVLSQSPAILSASPGETVTMTCRASSSVSFMYWLQQKPGSSPQPWIYATSNLASGVPARFSGSGSGTSYSLTITRVEAEDAATYYCQQWSFRPWTFGGGTKLEIK

SEQ ID NO: 98 - DNA, 318 bp, Mus musculus
caaattgttctctcccagtctccagcaatcctgtctgcatctccaggggagacggtcacaatgacttgcagggccagttcaagtgtaagtttcatgtactggctccagcagaagccaggttcctccccccaaccctggatttatgccacatccaacctggcttctggagtccctgctcgcttcagtggcagtgggtctgggacctcttactccctcacaatcaccagagtggaggctgaagatgctgccacttattactgtcaacagtggagttttagaccgtggacgttcggtggaggcaccaagctggaaatcaaa

SEQ ID NO: 99 - protein, 10 aa, Mus musculus
RASSSVSFMY

SEQ ID NO: 100 - protein, 7 aa, Mus musculus
ATSNLAS

SEQ ID NO: 101 - protein, 9 aa, Mus musculus
QQWSFRPWT

SEQ ID NO: 102 - protein, 117 aa, Mus musculus
DVQLQESGPGLVKPSQSLSLTCTVTGFSITSDYAWNWIRQFPGNKLEWMGYISYSGRTNYNPSLKSRFSITRDTSKNQFFLQLNSVTTEDTATYYCARSYDYWFPYWGQGTLVTVSA

SEQ ID NO: 103 - DNA, 351 bp, Mus musculus
gatgtgcagcttcaggagtcgggacctggcctggtgaaaccttctcagtctctgtccctcacctgcactgtcactggcttctcaatcaccagtgattatgcctggaactggatccggcagtttccaggaaacaaactggagtggatgggctacataagctacagtggtagaactaactacaacccatctctcaaaagtcgattctctatcactcgagacacatccaagaaccagttcttcctgcagttgaattctgtgactactgaggacacagccacatattactgtgcaagatcatatgattactggtttccttactggggccaagggactctggtcactgtctctgca

SEQ ID NO: 104 - protein, 16 aa, Mus musculus
YISYSGRTNYNPSLKS

SEQ ID NO: 105 - protein, 8 aa, Mus musculus
SYDYWFPY

SEQ ID NO: 106 - protein, 112 aa, Mus musculus
DVLMTQTPLSLPVSLGDQASISCRSSQSIVHSNGNTFLEWYLQKPGQSPKLLIYKVSNRFSGVPDRFSGSGSGTDFTLKISRVEAEDLGVYYCFQGSHIPVTFGAGTKLELK

SEQ ID NO: 107 - DNA, 336 bp, Mus musculus
gatgttttgatgacccaaactccactctccctgcctgtcagtcttggagatcaagcctccatctcttgcagatctagtcagagcattgtacatagtaatggaaacacctttttggaatggtacctgcagaaaccaggccagtctccaaagctcctgatctacaaagtttccaaccgattttctggggtcccagacaggttcagtggcagtggatcagggacagatttcacactcaagatcagcagagtggaggctgaggatctgggagtttattactgctttcaaggttcacatattccggtcacgttcggtgctgggaccaagctggagctgaaa

SEQ ID NO: 108 - protein, 16 aa, Mus musculus
RSSQSIVHSNGNTFLE

SEQ ID NO: 109 - protein, 7 aa, Mus musculus
KVSNRFS

SEQ ID NO: 110 - protein, 9 aa, Mus musculus
FQGSHIPVT

SEQ ID NO: 111 - protein, 117 aa, Mus musculus
EVQLQESGPGLVKPSQSLSLTCTVTGFSITSDYAWHWIRQFPGNKLEWMGFINYSGRTNYNPSLTSRISIIRDTSKNQFFLQLNSVTTEDTATYYCARSYDFWFGYWGQGTLVTVSA

SEQ ID NO: 112 - DNA, 351 bp, Mus musculus
gaggtccagctgcaggagtcgggacctggcctggtgaaaccttctcagtctctgtccctcacctgcactgtcactggcttctcaatcaccagtgattatgcctggcactggatccggcagtttccaggaaacaaactggagtggatgggcttcataaactacagtggtagaactaactacaacccatctctcacaagtcgaatctctatcattcgggacacatccaagaaccagttcttcctgcagttgaattctgtgactactgaggacacagccacatattactgtgcaagatcatatgatttctggtttggttattggggccaagggactctggtcactgtctctgca

SEQ ID NO: 113 - protein, 16 aa, Mus musculus
FINYSGRTNYNPSLTS

SEQ ID NO: 114 - protein, 8 aa, Mus musculus
SYDFWFGY

SEQ ID NO: 115 - protein, 112 aa, Mus musculus
NVLMTQSPLSLPVSLGDQASISCRSSQSIVHSNGNTYLEWYMQKPGQSPKLLIYTVSKRFSGVPDRFSGSGSGTDFTLKISRVEAEDLGVYYCFQGSHVPVTFGAGTKLELK

SEQ ID NO: 116 - DNA, 336 bp, Mus musculus
aatgttttgatgacccaaagtccactctccctgcctgtcagtcttggagatcaagcctccatctcttgcagatctagtcagagtattgtacatagtaatggaaacacctatttagaatggtatatgcagaaaccaggccagtctccaaagctcctgatctacacagtttccaaacgattttctggggtcccagacaggttcagtggcagtggatcagggacagatttcacactcaagatcagcagagtggaggctgaggatctgggagtttattattgctttcaaggttcacatgttccggtcacgttcggtgctgggaccaagctggagctgaaa

SEQ ID NO: 117 - protein, 16 aa, Mus musculus
RSSQSIVHSNGNTYLE

SEQ ID NO: 118 - protein, 7 aa, Mus musculus
TVSKRFS

SEQ ID NO: 119 - protein, 119 aa, Mus musculus
KVKLVESGGDLVKPGGSLKISCAASGFTFSNYAMSWIRQTPDKRLEWVATVSSGGPYTYYPDSVKGRFTISRDNAENTLYLQMSSLRSDDTAIYYCARQIYSDYDVTYWGQGTLVTVSA

SEQ ID NO: 120 - DNA, 357 bp, Mus musculus
aaagtgaagctggtggagtctgggggagacttagtgaagcctggagggtccctgaaaatctcctgtgcagcctctggattcactttcagtaactatgccatgtcttggattcgccagactccggacaagaggctggagtgggtcgcaaccgttagtagtggtggtccttacacctactatccagacagtgtgaaggggcgattcaccatctccagagacaatgccgaaaacaccctgtacctgcaaatgagcagtctgaggtctgatgacacggccatttattactgtgcaaggcagatctactctgattacgacgtcacttactggggccaagggactctggtcactgtctctgca

SEQ ID NO: 121 - protein, 106 aa, Mus musculus
QIVLSQSPAILSASPGETVTMTCRVSSSVSYMYWLQQKPGSSPKPWIYATSNLASGVPARFSGSGSGTSYSLTITRVEAEDAATYYCQQWSFRPWTFGGGTKLEIK

SEQ ID NO: 122 - DNA, 318 bp, Mus musculus
caaattgttctctcccagtctccagcaatcctgtctgcatctccaggggagacggtcacaatgacttgcagggtcagttcaagtgtaagttacatgtactggctccaacagaagccaggatcctcccccaaaccctggatttatgccacatccaacctggcttctggagtccctgctcgcttcagtggcagtgggtctgggacctcttactccctcacaatcaccagagtggaggctgaagatgctgccacttattactgtcagcagtggagttttagaccgtggacgttcggtggaggcaccaagctggaaatcaaa

SEQ ID NO: 123 - protein, 10 aa, Mus musculus
RVSSSVSYMY

SEQ ID NO: 124 - protein, 120 aa, Mus musculus
QVQLQQSGTELARPGASVRMSCKASGYTFRSHTMHWVKQRPGQGLEWIGYINPSTGYINYNQKFKDKATLTADKSSSTAYMQLSSLTSEDSAVYYCARSNYSYYYGMDYWGQGTSVTVSS

SEQ ID NO: 125 - DNA, 360 bp, Mus musculus
caggtccagctgcagcagtctgggactgaactggcaagacctggggcctcagtgaggatgtcctgcaaggcttctggctacacctttaggagtcacacgatgcactgggtaaaacagaggcctggacagggtctggaatggattggatacattaatcctagcactggttatattaattacaatcagaagttcaaggacaaggccacattgactgcagacaaatcctccagcacagcctacatgcaactgagcagcctgacatctgaggactctgcagtctattactgtgcaagaagtaactactcttattactatggtatggactactggggtcaaggaacctcagtcaccgtctcctca

SEQ ID NO: 126 - protein, 5 aa, Mus musculus
SHTMH

SEQ ID NO: 127 - protein, 17 aa, Mus musculus
YINPSTGYINYNQKFKD

SEQ ID NO: 128 - protein, 11 aa, Mus musculus
SNYSYYYGMDY

SEQ ID NO: 129 - protein, 107 aa, Mus musculus
DIVMTQSHKFMSTSVGDRVTITCKASQDVNTAVAWYQQKPGQSPKLLIYSASYRYTGVPDRFTGSGSGTDFTFTISSLQAEDLAVYYCQQHYNIPLTFGAGTKLELK

SEQ ID NO: 130 - DNA, 321 bp, Mus musculus
gacattgtgatgacccagtctcacaaattcatgtccacatcagtgggagacagggtcaccatcacctgcaaggccagtcaggatgtaaatactgctgtagcctggtatcaacagaaaccaggacaatctcctaaactactgatttactcggcatcctaccggtacactggggtccctgatcgcttcactggcagtggatctgggacggatttcactttcaccatcagcagtttacaggctgaagacctggcagtttattactgtcagcaacattataatattccgctcacgttcggtgctgggaccaagctggagctgaaa

SEQ ID NO: 131 - protein, 11 aa, Mus musculus
KASQDVNTAVA

SEQ ID NO: 132 - protein, 7 aa, Mus musculus
SASYRYT

SEQ ID NO: 133 - protein, 9 aa, Mus musculus
QQHYNIPLT

SEQ ID NO: 134 - protein, 120 aa, Mus musculus
QVQLQQSGTELARPGASVKMSCKASGYTFATYSIHWVKQRPGQGLEWIGYINPSSGYTNYNQKFRDKATLTADRSSNTAYMQLSSLTSEDSAVYYCARVYYTFYHAMDYWGQGTSVTVSS

SEQ ID NO: 135 - DNA, 360 bp, Mus musculus
caggtccagctgcagcagtctgggactgaactggcaagacctggggcctcagtgaagatgtcctgcaaggcttctggctacacctttgctacctactcgatacactgggtaaaacagaggcctgggcagggtctggaatggattggatacattaatcctagcagtggttatactaattacaatcagaagttcagggacaaggccacattgactgcagacagatcctccaacacagcctacatgcaactgagcagcctgacatctgaggactctgcagtctattactgtgcaagagtctactatactttttaccatgctatggactactggggtcaaggaacctcagtcaccgtctcctca

SEQ ID NO: 136 - protein, 6 aa, Mus musculus
ATYSIH

SEQ ID NO: 137 - protein, 17 aa, Mus musculus
YINPSSGYTNYNQKFRD

SEQ ID NO: 138 - protein, 11 aa, Mus musculus
VYYTFYHAMDY

SEQ ID NO: 139 - protein, 114 aa, Mus musculus
QMQLQESGPGLVKPSQSLSLTCTVTGYSITSDYAWNWIRQFPGNKLEWMGYISYSGRTSYNPSLKSRISITRDTSKNQFFLQLNSVTTEDTATYYCARHYGDYWGQGTTLTVSS

SEQ ID NO: 140 - DNA, 342 bp, Mus musculus
cagatgcagcttcaggagtcgggacctggcctggtgaaaccttctcagtctctgtccctcacctgcactgtcactggctactcaatcaccagtgattatgcctggaactggatccggcagtttccaggaaacaaactggagtggatgggctacataagctacagtggtaggactagctacaacccatctctcaaaagtcgaatctctatcactcgagacacatccaagaaccagttcttcctgcagttgaattctgtgactactgaggacacagccacatattactgtgcaagacactacggagactactggggccaaggcaccactctcacagtctcctca

SEQ ID NO: 141 - protein, 5 aa, Mus musculus
HYGDY

SEQ ID NO: 142 - protein, 107 aa, Mus musculus
DIVMTQSQKLMSTSVGDRVSVTCKASQNVGTNVAWYQQKPGQSPKALIYSASYRNSGVPDRFTGSGSGTDFTLTISNVQSEDLAEYFCQQFNTNPLTFGSGTKLEIK

SEQ ID NO: 143 - DNA, 321 bp, Mus musculus
gacattgtgatgactcagtctcaaaaactcatgtccacatcagtaggagacagggtcagcgtcacctgcaaggccagtcagaatgtgggtactaatgtagcctggtatcaacagaaaccagggcaatctcctaaagcactgatttactcggcatcctaccggaacagtggagtccctgatcgcttcacaggcagtggttctgggacagatttcactctcaccatcagcaatgtgcagtctgaagacttggcagagtatttctgtcagcaatttaacaccaatcctctcacgttcggctcggggacaaagttggaaataaaa

SEQ ID NO: 144 - protein, 11 aa, Mus musculus
KASQNVGTNVA

SEQ ID NO: 145 - protein, 7 aa, Mus musculus
SASYRNS

SEQ ID NO: 146 - protein, 9 aa, Mus musculus
QQFNTNPLT

SEQ ID NO: 147 - protein, 123 aa, Mus musculus
QVQLQQSGPQLLRPGASVKISCKASGFSFTNHWIHWVKQRPGQGLEWIGMIDPSDSETGLNQKFRDKATLTVDKSSSTAYMHLNSPTSEDSAVYYCARLGIHDGYYIYAMDFWGQGTSVTVSS

SEQ ID NO: 148 - DNA, 369 bp, Mus musculus
caggttcagctgcagcagtctgggcctcagctacttaggcctggggcttcagtgaagatatcctgcaaggcttctggtttctcattcaccaaccactggatacactgggtgaaacagaggcctggacaaggtcttgagtggattggcatgattgatccttccgatagtgaaactggcctcaatcagaagttcagggacaaggccacattgactgtagacaagtcctccagcacagcctacatgcacctcaacagcccgacatctgaggactctgcggtctattactgtgcaagattgggaatccatgatggttactacatctatgctatggacttttggggtcaaggaacctcagtcaccgtctcctca

SEQ ID NO: 149 - protein, 6 aa, Mus musculus
TNHWIH

SEQ ID NO: 150 - protein, 17 aa, Mus musculus
MIDPSDSETGLNQKFRD

SEQ ID NO: 151 - protein, 14 aa, Mus musculus
LGIHDGYYIYAMDF

SEQ ID NO: 152 - protein, 107 aa, Mus musculus
NIVMTQSPKSMSMSVGERVTLSCKASENVGTYVSWYQQKPEQSPKLLIYGASNRYTGVPDRFTGSGSATDFTLTISSVQAEDLADYHCGQSYSYPLTFGAGTKLELK

SEQ ID NO: 153 - DNA, 321 bp, Mus musculus
aacattgtaatgacccaatctcccaaatccatgtccatgtcagtaggagagagggtcaccttgagctgcaaggccagtgagaatgtgggtacttatgtatcctggtatcaacagaaaccagagcagtctcctaaactgctgatatacggggcatccaaccggtacactggggtccccgatcgcttcacaggcagtggatctgcaacagatttcactctgaccatcagcagtgtgcaggctgaagaccttgcagattatcactgtggacagagttacagctatccgctcacgttcggtgctgggaccaagctggagctgaaa

SEQ ID NO: 154 - protein, 11 aa, Mus musculus
KASENVGTYVS

SEQ ID NO: 155 - protein, 7 aa, Mus musculus
GASNRYT

SEQ ID NO: 156 - protein, 9 aa, Mus musculus
GQSYSYPLT

SEQ ID NO: 157 - protein, 114 aa, Mus musculus
EVQLQESGPGLVKPSQSLSLTCSVTGYSITSDYAWNWIRQFPGNKLEWMGYISYSGRTSYNPSLKSRISITRDTSKNQFFLQLISVTTEDTATYYCARYWGDYWGQGTTLTVSS

SEQ ID NO: 158 - DNA, 342 bp, Mus musculus
gaggtgcagcttcaggagtcgggacctggcctggtgaaaccttctcagtctctgtccctcacctgctctgtcactggctactcaatcaccagtgattatgcctggaactggatccggcagtttccaggaaacaagctggagtggatgggctacataagttacagtggtagaactagctacaacccatctctcaaaagtcgaatctctatcactcgagacacatccaagaaccagttcttcctgcagttgatttctgtgactactgaggacacagccacatattattgtgcaagatattggggcgactactggggccaaggcaccactctcacagtctcctca

SEQ ID NO: 159 - protein, 107 aa, Mus musculus
DIVMTQSQKFISTSIGDRVSVTCKASQDVGGHVAWFQQRPGQSPKPLIYSATFRHSGVPDRFTGSGSGTDFTLTISNLQSEDLAEYVCLQYNSNPLTFGPGTKLELK

SEQ ID NO: 160 - DNA, 321 bp, Mus musculus
gacattgtgatgacccagtctcaaaaattcatctccacatcaataggagacagggtcagcgtcacctgcaaggccagtcaggatgtgggtggacatgtggcctggtttcaacagagacccgggcaatctcctaaacctctgatttattcggcaaccttccggcacagtggagtccctgatcgcttcacgggcagtggatctgggacagatttcactctcaccatcagtaatctacagtctgaggacttggcagaatatgtctgtctgcaatataacagtaatccactcacgttcggtcctgggaccaagctggagctgaaa

SEQ ID NO: 161 - protein, 11 aa, Mus musculus
KASQDVGGHVA

SEQ ID NO: 162 - protein, 7 aa, Mus musculus
SATFRHS

SEQ ID NO: 163 - protein, 114 aa, Mus musculus
DVQLQESGPGLVKPSQSLSLTCTVTGYSITSDYAWNWIRQFPGNKLEWMGYISYSGRTSYNPYLKSRISITRDTSKNQFFLQLNSVTTEDTATYYCARYWGDYWGQGTTLTVSS

SEQ ID NO: 164 - DNA, 342 bp, Mus musculus
gatgtgcagcttcaggagtcgggacctggcctggtgaaaccttctcagtctctgtccctcacctgcactgtcactggctactcaatcaccagtgattatgcctggaactggatccggcagtttccaggaaacaaactggagtggatgggctacataagctacagtggtcgcactagctacaacccatatctcaaaagtcgaatttctatcactcgagacacatccaagaaccagttcttcctgcagttgaattctgtgactactgaggacacagccacatattactgtgcaagatattggggcgactactggggccaaggcaccactctcacagtctcctca

SEQ ID NO: 165 - protein, 16 aa, Mus musculus
YISYSGRTSYNPYLKS

SEQ ID NO: 166 - protein, 107 aa, Mus musculus
DIVMTQSQKFMSTSVGDRVSVTCKASQNVGTNVAWYKQKPGQSPKALIYSASYRHSGVPDRFTGSGSGTDFTLTISNVQSEDLAEYFCLQYNSNPLTFGAGTKLELK

SEQ ID NO: 167 - DNA, 321 bp, Mus musculus
gacattgtgatgacccagtctcaaaaattcatgtccacatcagtaggagacagggtcagcgtcacctgcaaggccagtcagaatgtgggtactaatgtagcctggtataaacagaaaccagggcaatctcctaaagcactgatttactcggcatcctaccggcacagtggagtccctgatcgcttcacaggcagtggatctgggacagatttcactctcaccatcagcaatgtgcagtctgaagacttggcagagtatttctgtctgcaatataacagcaatcctctcacgttcggtgctgggaccaagctggagctgaaa

SEQ ID NO: 168 - protein, 7 aa, Mus musculus
SASYRHS

SEQ ID NO: 169 - protein, 114 aa, Mus musculus
DVQLQESGPGLVKPSQSLSLTCTVTGYSITSDYAWNWIRQFPGNKLEWMGYISYSGRTSYNPSLKSRISITRDTSKNQFFLQLNSVTAEDTATYYCARYWGDYWGQGTTLTVSS

SEQ ID NO: 170 - DNA, 342 bp, Mus musculus
gatgtgcagcttcaggagtcgggacctggcctggtgaaaccttctcagtctctgtccctcacctgcactgtcactggctactcaatcaccagtgattatgcctggaactggatccggcagtttccaggaaacaaactggagtggatgggctacataagctacagtggtcgcactagctacaacccatctctcaaaagtcgaatctctatcactcgagacacatccaagaaccagttcttcctgcagttgaattctgtgactgctgaggacacagccacatattactgtgcaagatattggggcgactactggggccaaggcaccactctcacagtctcctca

SEQ ID NO: 171 - protein, 107 aa, Mus musculus
DIVMTQSQKFMSTSVGDRVSVTCKASQNVGTNVAWFQQKPGQSPKALIYSTSYRSSGVPDRFTGSGSGTDFTLTISNVQSEDLAEYFCQQFNSNPLTFGGGTKLELK

SEQ ID NO: 172 - DNA, 321 bp, Mus musculus
gacattgtgatgacacagtctcaaaaattcatgtccacatcagtaggagacagggtcagcgtcacctgcaaggccagtcagaatgtgggtactaatgtagcctggtttcaacagaaaccagggcaatctcctaaagcactgatttactcgacatcctaccggtccagtggagtccctgatcgcttcacaggcagtggatctgggacagatttcactctcaccatcagcaatgtgcagtctgaagacttggcagagtacttctgtcagcaatttaacagcaatcctctcacgttcggaggggggaccaagctggagctgaaa

SEQ ID NO: 173 - protein, 7 aa, Mus musculus
STSYRSS

SEQ ID NO: 174 - protein, 9 aa, Mus musculus
QQFNSNPLT

SEQ ID NO: 175 - protein, 114 aa, Homo sapiens
QMQLQESGPGLVKPSETLSLTCTVSGYSITSDYAWNWIRQPPGKGLEWIGYISYSGRTSYNPSLKSRVTISRDTSKNQFSLKLSSVTAADTAVYYCARHYGDYWGQGTLVTVSS

SEQ ID NO: 176 - DNA, 342 bp, Homo sapiens
cagatgcagctgcaagagtctggacctggactggtcaagcccagcgagacactgagcctgacctgtaccgtgtccggctacagcatcacaagcgactacgcctggaactggatcagacagcctcctggcaaaggcctcgagtggatcggctacatcagctacagcggcagaaccagctacaaccccagcctgaagtccagagtgaccatcagcagagacaccagcaagaaccagttctccctgaagctgagcagcgtgacagccgccgatacagccgtgtactactgcgctagacactacggcgattactggggccagggaaccctggtcacagtgtcatct

SEQ ID NO: 177 - protein, 114 aa, Homo sapiens
QLQLQESGPGLVKPSETLSLTCTVSGYSITSDYAWNWIRQPPGKGLEWIGYISYSGRTSYNPSLKSRVTISRDTSKNQFSLKLSSVTAADTAVYYCARHYGDYWGQGTLVTVSS

SEQ ID NO: 178 - DNA, 342 bp, Homo sapiens
cagctccagctgcaagagtctggacctggactggtcaagcccagcgagacactgagcctgacctgtaccgtgtccggctacagcatcacaagcgactacgcctggaactggatcagacagcctcctggcaaaggcctcgagtggatcggctacatcagctacagcggcagaaccagctacaaccccagcctgaagtccagagtgaccatcagcagagacaccagcaagaaccagttctccctgaagctgagcagcgtgacagccgccgatacagccgtgtactactgcgctagacactacggcgattactggggccagggaaccctggtcacagtgtcatct

SEQ ID NO: 179 - protein, 114 aa, Homo sapiens
QLQLQESGPGLVKPSETLSLTCTVSGYSITSDYAWNWIRQPPGKGLEWIGYISYSGRTSYNPSLKSRVTISVDTSKNQFSLKLSSVTAADTAVYYCARHYGDYWGQGTLVTVSS

SEQ ID NO: 180 - DNA, 342 bp, Homo sapiens
cagctccagctgcaagagtctggacctggactggtcaagcccagcgagacactgagcctgacctgtaccgtgtccggctacagcatcacaagcgactacgcctggaactggatcagacagcctcctggcaaaggcctcgagtggatcggctacatcagctacagcggcagaaccagctacaaccccagcctgaagtccagagtgaccatcagcgtagacaccagcaagaaccagttctccctgaagctgagcagcgtgacagccgccgatacagccgtgtactactgcgctagacactacggcgattactggggccagggaaccctggtcacagtgtcatct

SEQ ID NO: 181 - protein, 120 aa, Homo sapiens
QVQLVQSGAEVKKPGSSVKVSCKASGYTFATYSIHWVRQAPGQGLEWMGYINPSSGYTNYNQKFQGRVTLTADKSTSTAYMELSSLRSEDTAVYYCARVYYTFYHAMDYWGQGTTVTVSS

SEQ ID NO: 182 - DNA, 360 bp, Homo sapiens
caggttcagctggttcagtctggcgccgaagtgaagaaacctggcagcagcgtgaaggtgtcctgcaaggctagcggctacaccttcgccacctacagcatccactgggtccgacaggctccaggacagggacttgagtggatgggctacatcaaccccagctctggctacaccaactacaaccagaaattccagggccgcgtgaccctcacagccgacaagtctacaagcaccgcctacatggaactgagcagcctgagaagcgaggacaccgccgtgtactactgcgccagagtgtactacacattctaccacgccatggactactggggccagggcacaacagtgaccgttagctct

SEQ ID NO: 183 - protein, 17 aa, Homo sapiens
YINPSSGYTNYNQKFQG

SEQ ID NO: 184 - protein, 120 aa, Homo sapiens
QVQLVQSGAEVKKPGSSVKVSCKASGYTFATYSIHWVRQAPGQGLEWMGYINPSSGYTNYNQKFQGRVTLTADESTSTAYMELSSLRSEDTAVYYCARVYYTFYHAMDYWGQGTTVTVSS

SEQ ID NO: 185 - DNA, 360 bp, Homo sapiens
caggttcagctggttcagtctggcgccgaagtgaagaaacctggcagcagcgtgaaggtgtcctgcaaggctagcggctacaccttcgccacctacagcatccactgggtccgacaggctccaggacagggacttgagtggatgggctacatcaaccccagctctggctacaccaactacaaccagaaattccagggccgcgtgaccctcacagccgacgagtctacaagcaccgcctacatggaactgagcagcctgagaagcgaggacaccgccgtgtactactgcgccagagtgtactacacattctaccacgccatggactactggggccagggcacaacagtgaccgttagctct

SEQ ID NO: 186 - protein, 120 aa, Homo sapiens
QVQLVQSGAEVKKPGSSVKVSCKASGYTFATYSIHWVRQAPGQGLEWMGYINPSSGYTNYNQKFQGRVTITADKSTSTAYMELSSLRSEDTAVYYCARVYYTFYHAMDYWGQGTTVTVSS

SEQ ID NO: 187 - DNA, 360 bp, Homo sapiens
caggttcagctggttcagtctggcgccgaagtgaagaaacctggcagcagcgtgaaggtgtcctgcaaggctagcggctacaccttcgccacctacagcatccactgggtccgacaggctccaggacagggacttgagtggatgggctacatcaaccccagctctggctacaccaactacaaccagaaattccagggccgcgtgaccatcacagccgacaagtctacaagcaccgcctacatggaactgagcagcctgagaagcgaggacaccgccgtgtactactgcgccagagtgtactacacattctaccacgccatggactactggggccagggcacaacagtgaccgttagctct

SEQ ID NO: 188 - protein, 120 aa, Homo sapiens
QVQLVQSGAEVKKPGSSVKVSCKASGYTFATYSIHWVRQAPGQGLEWMGYINPSSGYTNYNQKFQGRVTITADESTSTAYMELSSLRSEDTAVYYCARVYYTFYHAMDYWGQGTTVTVSS

SEQ ID NO: 189 - DNA, 360 bp, Homo sapiens
caggttcagctggttcagtctggcgccgaagtgaagaaacctggcagcagcgtgaaggtgtcctgcaaggctagcggctacaccttcgccacctacagcatccactgggtccgacaggctccaggacagggacttgagtggatgggctacatcaaccccagctctggctacaccaactacaaccagaaattccagggccgcgtgaccatcacagccgacgagtctacaagcaccgcctacatggaactgagcagcctgagaagcgaggacaccgccgtgtactactgcgccagagtgtactacacattctaccacgccatggactactggggccagggcacaacagtgaccgttagctct

SEQ ID NO: 190 - protein, 120 aa, Homo sapiens
QVQLVQSGAEVKKPGSSVKVSCKASGYTFRSHTMHWVRQAPGQGLEWMGYINPSTGYINYNQKFQGRVTLTADKSTSTAYMELSSLRSEDTAVYYCARSNYAYYYGMDYWGQGTTVTVSS

SEQ ID NO: 191 - DNA, 360 bp, Homo sapiens
caggttcagctggttcagtctggcgccgaagtgaagaaacctggcagcagcgtgaaggtgtcctgcaaggctagcggctacaccttcagatcccacaccatgcactgggtccgacaggctccaggacagggacttgagtggatgggctacatcaaccccagcaccggctatatcaactacaaccagaaattccagggccgcgtgaccctcacagccgacaagtctacaagcaccgcctacatggaactgagcagcctgagaagcgaggacaccgccgtgtactactgcgccagaagcaactacgcctactactacggcatggactactggggccagggcaccacagtgacagtctcttct

SEQ ID NO: 192 - protein, 17 aa, Homo sapiens
YINPSTGYINYNQKFQG

SEQ ID NO: 193 - protein, 120 aa, Homo sapiens
QVQLVQSGAEVKKPGSSVKVSCKASGYTFRSHTMHWVRQAPGQGLEWMGYINPSTGYINYNQKFQGRVTLTADESTSTAYMELSSLRSEDTAVYYCARSNYAYYYGMDYWGQGTTVTVSS

SEQ ID NO: 194 - DNA, 360 bp, Homo sapiens
caggttcagctggttcagtctggcgccgaagtgaagaaacctggcagcagcgtgaaggtgtcctgcaaggctagcggctacaccttcagatcccacaccatgcactgggtccgacaggctccaggacagggacttgagtggatgggctacatcaaccccagcaccggctatatcaactacaaccagaaattccagggccgcgtgaccctcacagccgacgagtctacaagcaccgcctacatggaactgagcagcctgagaagcgaggacaccgccgtgtactactgcgccagaagcaactacgcctactactacggcatggactactggggccagggcaccacagtgacagtctcttct

SEQ ID NO: 195 - protein, 120 aa, Homo sapiens
QVQLVQSGAEVKKPGSSVKVSCKASGYTFRSHTMHWVRQAPGQGLEWMGYINPSTGYINYNQKFQGRVTITADKSTSTAYMELSSLRSEDTAVYYCARSNYAYYYGMDYWGQGTTVTVSS

SEQ ID NO: 196 - DNA, 360 bp, Homo sapiens
caggttcagctggttcagtctggcgccgaagtgaagaaacctggcagcagcgtgaaggtgtcctgcaaggctagcggctacaccttcagatcccacaccatgcactgggtccgacaggctccaggacagggacttgagtggatgggctacatcaaccccagcaccggctatatcaactacaaccagaaattccagggccgcgtgaccatcacagccgacaagtctacaagcaccgcctacatggaactgagcagcctgagaagcgaggacaccgccgtgtactactgcgccagaagcaactacgcctactactacggcatggactactggggccagggcaccacagtgacagtctcttct

SEQ ID NO: 197 - protein, 120 aa, Homo sapiens
QVQLVQSGAEVKKPGSSVKVSCKASGYTFRSHTMHWVRQAPGQGLEWMGYINPSTGYINYNQKFQGRVTITADESTSTAYMELSSLRSEDTAVYYCARSNYAYYYGMDYWGQGTTVTVSS

SEQ ID NO: 198 - DNA, 360 bp, Homo sapiens
caggttcagctggttcagtctggcgccgaagtgaagaaacctggcagcagcgtgaaggtgtcctgcaaggctagcggctacaccttcagatcccacaccatgcactgggtccgacaggctccaggacagggacttgagtggatgggctacatcaaccccagcaccggctatatcaactacaaccagaaattccagggccgcgtgaccatcacagccgacgagtctacaagcaccgcctacatggaactgagcagcctgagaagcgaggacaccgccgtgtactactgcgccagaagcaactacgcctactactacggcatggactactggggccagggcaccacagtgacagtctcttct

SEQ ID NO: 199 - protein, 107 aa, Homo sapiens
DIQMTQSPSSLSASVGDRVTITCRASQNVGTNVAWYQQKPGKAPKALIYSASYRESGVPSRFSGSGSGTDFTLTISSLQPEDFATYFCQQFNTNPLTFGGGTKVEIK

SEQ ID NO: 200 - DNA, 321 bp, Homo sapiens
gacatccagatgacacagagccctagcagcctgtctgccagcgtgggagacagagtgaccatcacctgtagagccagccagaacgtgggcacaaacgtggcctggtatcagcagaagcctggcaaggctcccaaggcgctgatctacagcgccagctacagagagagcggcgtgccatctagattcagcggctctggctctggcaccgacttcaccctgacaatctctagcctgcagcctgaggacttcgctacctacttctgccagcagttcaacacaaaccctctgaccttcggcggaggcaccaaggtggaaatcaag

SEQ ID NO: 201 - protein, 11 aa, Homo sapiens
RASQNVGTNVA

SEQ ID NO: 202 - protein, 7 aa, Homo sapiens
SASYRES

SEQ ID NO: 203 - protein, 107 aa, Homo sapiens
DIQMTQSPSSLSASVGDRVTITCRASQNVGTNVAWYQQKPGKAPKLLIYSASYRESGVPSRFSGSGSGTDFTLTISSLQPEDFATYFCQQFNTNPLTFGGGTKVEIK

SEQ ID NO: 204 - DNA, 321 bp, Homo sapiens
gacatccagatgacacagagccctagcagcctgtctgccagcgtgggagacagagtgaccatcacctgtagagccagccagaacgtgggcacaaacgtggcctggtatcagcagaagcctggcaaggctcccaagctgctgatctacagcgccagctacagagagagcggcgtgccatctagattcagcggctctggctctggcaccgacttcaccctgacaatctctagcctgcagcctgaggacttcgctacctacttctgccagcagttcaacacaaaccctctgaccttcggcggaggcaccaaggtggaaatcaag

SEQ ID NO: 205 - protein, 107 aa, Homo sapiens
DIQMTQSPSSLSASVGDRVTITCRASQNVGTNVAWYQQKPGKAPKALIYSASYRQSGVPSRFSGSGSGTDFTLTISSLQPEDFATYFCQQFNTNPLTFGGGTKVEIK

SEQ ID NO: 206 - DNA, 321 bp, Homo sapiens
gacatccagatgacacagagccctagcagcctgtctgccagcgtgggagacagagtgaccatcacctgtagagccagccagaacgtgggcacaaacgtggcctggtatcagcagaagcctggcaaggctcccaaggcgctgatctacagcgccagctacagacagagcggcgtgccatctagattcagcggctctggctctggcaccgacttcaccctgacaatctctagcctgcagcctgaggacttcgctacctacttctgccagcagttcaacacaaaccctctgaccttcggcggaggcaccaaggtggaaatcaag

SEQ ID NO: 207 - protein, 7 aa, Homo sapiens
SASYRQS

SEQ ID NO: 208 - protein, 107 aa, Homo sapiens
EIVMTQSPATLSVSPGERATLSCRASQNVGTNVAWYQQKPGQAPRALIYSASYRESGIPARFSGSGSGTEFTLTISSLQSEDFAVYFCQQFNTNPLTFGGGTKVEIK

SEQ ID NO: 209 - DNA, 321 bp, Homo sapiens
gagatcgtgatgacacagagccccgccacactgagtgtgtctccaggcgaaagagctaccctgagctgtagagcctctcagaacgtgggcacaaacgtggcctggtatcagcagaagcctggacaggctcccagagcgctgatctacagcgccagctacagagagtctggcatccctgctagattcagcggctctggctctggcaccgagttcaccctgacaatcagcagcctgcagagcgaggacttcgccgtgtacttctgccagcagttcaacacaaaccctctgaccttcggcggaggcaccaaggtggaaatcaag

SEQ ID NO: 210 - protein, 107 aa, Homo sapiens
EIVMTQSPATLSVSPGERATLSCRASQNVGTNVAWYQQKPGQAPRLLIYSASYRESGIPARFSGSGSGTEFTLTISSLQSEDFAVYFCQQFNTNPLTFGGGTKVEIK

SEQ ID NO: 211 - DNA, 321 bp, Homo sapiens
gagatcgtgatgacacagagccccgccacactgagtgtgtctccaggcgaaagagctaccctgagctgtagagcctctcagaacgtgggcacaaacgtggcctggtatcagcagaagcctggacaggctcccagactgctgatctacagcgccagctacagagagtctggcatccctgctagattcagcggctctggctctggcaccgagttcaccctgacaatcagcagcctgcagagcgaggacttcgccgtgtacttctgccagcagttcaacacaaaccctctgaccttcggcggaggcaccaaggtggaaatcaag

SEQ ID NO: 212 - protein, 107 aa, Homo sapiens
EIVMTQSPATLSVSPGERATLSCRASQNVGTNVAWYQQKPGQAPRALIYSASYRQSGIPARFSGSGSGTEFTLTISSLQSEDFAVYFCQQFNTNPLTFGGGTKVEIK

SEQ ID NO: 213 - DNA, 321 bp, Homo sapiens
gagatcgtgatgacacagagccccgccacactgagtgtgtctccaggcgaaagagctaccctgagctgtagagcctctcagaacgtgggcacaaacgtggcctggtatcagcagaagcctggacaggctcccagagcgctgatctacagcgccagctacagacagtctggcatccctgctagattcagcggctctggctctggcaccgagttcaccctgacaatcagcagcctgcagagcgaggacttcgccgtgtacttctgccagcagttcaacacaaaccctctgaccttcggcggaggcaccaaggtggaaatcaag

SEQ ID NO: 214 - protein, 107 aa, Homo sapiens
DIQMTQSPSSLSASVGDRVTITCRASQDVNTAVAWYQQKPGKAPKLLIYSASYRYTGVPSRFSGSGSGTDFTLTISSLQPEDFATYYCQQHYNIPLTFGGGTKVEIK

SEQ ID NO: 215 - DNA, 321 bp, Homo sapiens
gacatccagatgacacagagccctagcagcctgtctgccagcgtgggagacagagtgaccatcacctgtagagccagccaggacgtgaacacagccgtggcttggtatcagcagaagcctggcaaggcccctaagctgctgatctacagcgccagctacagatacaccggcgtgccctctagattcagcggctctggctctggcaccgacttcaccctgacaatctctagcctgcagcctgaggacttcgccacctactactgccagcagcactacaacatccctctgaccttcggcggaggcaccaaggtggaaatcaag

SEQ ID NO: 216 - protein, 11 aa, Homo sapiens
RASQDVNTAVA